European Patent Application EP 4 226 936 A2, published August 16, 2023. Title: NON-NEUROINVASIVE VIRUSES AND USES THEREOF. Applicant: Northwestern University. The sequence listing filed with the application follows.

SEQUENCE LISTING (36 sequences)

SEQ ID NO: 1 - DNA, 34 bp, synthetic construct
  misc_feature 1..34: note = DNA Primer
  source 1..34: mol_type = other DNA
gggaattccatatgggcagcagccatcaccatca

SEQ ID NO: 2 - DNA, 30 bp, synthetic construct
  misc_feature 1..30: note = DNA Primer
  source 1..30: mol_type = other DNA
ttcaagacaaggtccccgggcctagggatc

SEQ ID NO: 3 - DNA, 30 bp, synthetic construct
  misc_feature 1..30: note = DNA Primer
  source 1..30: mol_type = other DNA
ctagggatccatggaagcactggttcgtgc

SEQ ID NO: 4 - DNA, 29 bp, synthetic construct
  misc_feature 1..29: note = DNA Primer
  source 1..29: mol_type = other DNA
gtggctggcgcgtcggatcttcgaagatc

SEQ ID NO: 5 - DNA, 94 bp, synthetic construct
  misc_feature 1..94: note = DNA Primer
  source 1..94: mol_type = other DNA
ctcgccgagaacctggccggcctggcgctgtggcgcctgcgccacgcctgggccgcgggcacggccccgctgaggatgacgacgataagtaggg

SEQ ID NO: 6 - DNA, 97 bp, synthetic construct
  misc_feature 1..97: note = DNA Primer
  source 1..97: mol_type = other DNA
gtcgccgttgacgacccccaggagctccagcagcggggccgtgcccgcggcccaggcgtggcgcaggcgccacaaccaattaaccaattctgattag

SEQ ID NO: 7 - DNA, 88 bp, synthetic construct
  misc_feature 1..88: note = DNA Primer
  source 1..88: mol_type = other DNA
gtcggctgcacggcggtcgtcggcggcgtcgtgcaccgcctcctcgccgcctacgggcccgggctgaggatgacgacgataagtaggg

SEQ ID NO: 8 - DNA, 91 bp, synthetic construct
  misc_feature 1..91: note = DNA Primer
  source 1..91: mol_type = other DNA
cgcgacgtccgtgtaggcgcgcacgtagtccagcccgggcccgtaggcggcgaggaggcggtgcaccaaccaattaaccaattctgattag

SEQ ID NO: 9 - DNA, 85 bp, synthetic construct
  misc_feature 1..85: note = DNA Primer
  source 1..85: mol_type = other DNA
ctcgaccacacgcaggtggacgccacgggcgtgtgggaggcggtggcggccagcgcctcgccgaggatgacgacgataagtaggg

SEQ ID NO: 10 - DNA, 88 bp, synthetic construct
  misc_feature 1..88: note = DNA Primer
  source 1..88: mol_type = other DNA
cgcggtcacgagcgcctccacgacctgcagcggcgaggcgctggccgccaccgcctcccacaccaaccaattaaccaattctgattag

SEQ ID NO: 11 - DNA, 94 bp, synthetic construct
  misc_feature 1..94: note = DNA Primer
  source 1..94: mol_type = other DNA
gacctcctcgagcgcgccgtgctggaccgcgcgccccgcctgacggccgcgcaggctgccgtcggctgcacgaggatgacgacgataagtaggg

SEQ ID NO: 12 - DNA, 97 bp, synthetic construct
  misc_feature 1..97: note = DNA Primer
  source 1..97: mol_type = other DNA
gaggcggtgcacgacgccgccgacgaccgccgtgcagccgacggcagcctgcgcggccgtcaggcggggcgccaaccaattaaccaattctgattag

SEQ ID NO: 13 - DNA, 97 bp, synthetic construct
  misc_feature 1..97: note = DNA Primer
  source 1..97: mol_type = other DNA
ggggacgtgacggcggcgctggggctccccgagaagggcgtggaggccgtggtgcgcgcttgcatggcgccgcgcaggatgacgacgataagtaggg

SEQ ID NO: 14 - DNA, 100 bp, synthetic construct
  misc_feature 1..100: note = DNA Primer
  source 1..100: mol_type = other DNA
gcgcgccgcgcccacgtgctccgtgggcgggcgcggcgccatgcaagcgcgcaccacggcctccacgcccttctccaaccaattaaccaattctgattag

SEQ ID NO: 15 - DNA, 88 bp, synthetic construct
  misc_feature 1..88: note = DNA Primer
  source 1..88: mol_type = other DNA
ctgccgctggcgttggcggtgcgccagatgcagaacgagggcctggcgcagctgacgcgcgcgctcaggatgacgacgataagtaggg

SEQ ID NO: 16 - DNA, 91 bp, synthetic construct
  misc_feature 1..91: note = DNA Primer
  source 1..91: mol_type = other DNA
gaagaactcgtcggcgatcgtgagggcaaagagcgcgcgcgtcagctgcgccaggccctcgttctgcaaccaattaaccaattctgattag

SEQ ID NO: 17 - DNA, 88 bp, synthetic construct
  misc_feature 1..88: note = DNA Primer
  source 1..88: mol_type = other DNA
aacccgacgctgcgcgagcagttcgccgaggcggcgcgggccgtggccgcggcggcgctggtgcccaggatgacgacgataagtaggg

SEQ ID NO: 18 - DNA, 91 bp, synthetic construct
  misc_feature 1..91: note = DNA Primer
  source 1..91: mol_type = other DNA
cgtgcgcggcgtggcgttgacctcgcccacgggcaccagcgccgccgcggccacggcccgcgccgccaaccaattaaccaattctgattag

SEQ ID NO: 19 - DNA, 92 bp, synthetic construct
  misc_feature 1..92: note = DNA Primer
  source 1..92: mol_type = other DNA
ccgaggcggcgcgggccgtggacgaggcggcgctggtgcccgtgggcgagacgcaggtggacgccacgggaggatgacgacgataagtaggg

SEQ ID NO: 20 - DNA, 95 bp, synthetic construct
  misc_feature 1..95: note = DNA Primer
  source 1..95: mol_type = other DNA
gaggcgctggcctgcaccgcctcccacacgcccgtggcgtccacctgcgtctcgcccacgggcaccagcgcaaccaattaaccaattctgattag

SEQ ID NO: 21 - DNA, 10 bp, synthetic construct
  misc_feature 1..10: note = Linker sequence
  source 1..10: mol_type = other DNA
gsgsgsgsgs

SEQ ID NO: 22 - protein, 424 aa, Suid herpesvirus 1
MEALVRALEEADHAVATVVQSRILEFFMAAGRETPAGVRGLWARALRLACRAYVETGTCEAAVLAENLAGLALWRLRHDWDEGTAPLLELLGVVNGDDTTAALTEAGLRTSAEFGPDAMFRLVSEWCAAFDEALAGARSADDVLAAPRVVPPEQTARALVQPRFATLYDMDFVQDGLRYVAQHTNWALPLALAVRQMQNEGLKPLTRALFAHGDAYVRELRPGTVARRLRTDQGVLALLDPGAQAVHVAAAADLDHTQVDATGVWEAVQASASPLQVVEALVTAGFTRRHCDLLERAVLDRAPRLTDAQRAVGCTAVVGGVVHRLLDDYGPGLDYVRAYTDVADTLEPLYGDVTAALGLPEKGVEHVVRHCMAPRPPTEHVGAARAALLREVAAAERRAGLAHSAAREALNTWLAFRAQSRWGL

SEQ ID NO: 23 - protein, 537 aa, Bovine herpesvirus 1
MSGDPVRALWAALERLDGEVAGPAALAEARAAVSEFLLASGPSSLDFVAPRWAALQRAACRAYERLHTPDAALLAENLPGLVLWRLPGAARDTADFMAGVRDLANSMIAEAPLGYLAAARLRATAAFGPVNMQRVVVEWASLFLEIYAREDAACVGVLGPDPACRSPAGSAAVIRPLLQSRFRLLYDMPFFQAGLSALAHAANWKVPMAAVARRAADAAAPPLARALFAVALVDEYFPEPDDEDTAPGLAEAFAEIADLVPPEALVPAGEANAFARSSHDVRVSAALAYRDPFVRGAAAGSVAARVRADAGLLADDTLLGRDAVAVHAGAVVRLLERAAARATPAALGRVAEHAAAVWDAVQASATPDQAVETLAAAGFTPGTCAMLERAVLAQLSRPEPRAPADVLQAVGCVAVAGGVLFKLFDAYGPSADYLAHYTATIANLHPYYADVLPLLGLPDGGLEQTIRHCMAPRPRTDYVAAIRAALAAEAAAADKRAASASARAAVENSGDRAAAGAAAREALLTWFDLRASERWGV

SEQ ID NO: 24 - protein, 541 aa, Equine herpesvirus 4
MAREDWSMRALVNTLAGLLGETDTDVTSMEPAMLMVLKSSISEFFLSTDTVSVEEAAELFPRLQFLACRAYAASHTPEAAMLAENLSGLVLWRIHQNWTDRETEAVDQMFVLLEIMNGESGVYMLSNNNLRISAKYGPSNMHLMVSTWLGTFRNVMLSIANTTPDAMFNARRIEAIEEFSKPLVHKRFDLIYDMPFVQEGLRIVAAKINWLLPFGLIAKRSKDTSMAPLTRALFLLSLVDSYFPKGTATNSSMKALTIYFREIVRNIDNSAFVPVTEVNATPRTAYEVRVSSAIVHQNPYVTDTKAGMVAERVRTDAEILSSGALLSSGALSAHVTAVAKLLAFNDQNDTSSVARARVAEHASNTWEAIQASTTPAQVVEALVTAGFTSTHCGILERVVVDYFTRLRSTAESRPGQDNSLDYAQQVVGCVSIVGGVVFRLLMSYGFGLDYIRDYTTTISTLEPVYNELLLALGLADKGVEQTLRRSMAPRPYMNYISAARAALDNELLIVEKRTTGPGTHSAARESLLTWFDFRARDRWGV

SEQ ID NO: 25 - protein, 540 aa, Felid herpesvirus 1
MDNSGPLMTLVASLEGLVGVASDRLTQDGVLRIKSMISEFFLSTDSIELRDTQRLWAKLQKLACDAYLHTRSPETAFLAENLPGLIFWRFKHDWTESPINDLTDISTLLDVMNDEECMACITTAGLRVSSFLGPSNIYRLVSEWIVLFKEIYLGVLNKTPSDALNEPPISSLDKFSEPLVSKKFELLYGMPFVQEGLRVIAIRANWLVQFGVMVQRTRDSTLTPLTRALYMLALVDEYFQDIEQTSTYTTLVRDFLELTQEIDEGALVPLQAANLSPRTAYEVRISSAIAHQNPFITNPQPGTVTVRLRTDPEILTERHLNLEALLIHVTAIIRLLDSKDITYEDGSNTIWNYVVECTTNTWEVIQASTNPHQAIEALIQAGFTSFHCSMLERAISDKFSKARISNINRHSIQRPLLDEAQQAIGCVAMVGSLIFKLVTHYGNGLDYIRHYTTTLADLPLVYGDLLDSLGLPNGSVEQIIRHCMAPKPYIDYITNSRVVFETELNLVDQRVVTVEGNTHNAARESLLMWFDFKARDLWGI

SEQ ID NO: 26 - protein, 553 aa, Cercopithecine herpesvirus 9
MWFDVFCIVHPTVDIMETAITQNLLNDLKSLSSKDDSSETIWPPEKVETARISIVKFLRSTQEIPLENTLWTELHKVICNVYAHTFLIEASFLAENLPGLIFWKLESHCTQNVMQHMETLKQLCNNIQSRETLQRLTLHSLRTSAKLGPVSINSLVTDWINMFEVAVRDINEATKLPFLYARQGMVESAVAALTHQRFALLYDMPIVQDGLRILTQRASWLIPFTIMWSHIQSDSFTPLTKCLFIINLADEYFDDTPVSYLTDLFNDNIIHVKDIAFVPIEEAIVQATTVHGARINAALAHQNLSIRQTQPGTATHRLRVDVNIWDNNILSLSAPGIHIDGLLHLITTDPTAETTAGAAVAECVRVAWERVQASTSPNSLVLALLEAGFTRYTCKLLRKFVTHCTLGLHSLYDTHITHEVCKLTDFQQTIGCVSLVGGLAYQLLETYAPTAHYVSTYTHILSETEKRYETLIPALGLPPGGLGQIMRRCFAPRPLISSIQLARKTLVEEINTAETRKTVLHLQHTRETQPGARVTREAILTWFDFRMESRWGI

SEQ ID NO: 27 - protein, 547 aa, Varicella zoster virus
MEEPICYDTQKLLDDLSNLKVQEADNERPWSPEKTEIARVKVVKFLRSTQKIPAKHFIQIWEPLHSNICFVYSNTFLAEAAFTAENLPGLLFWRLDLDWTIEEPGNSLKILTQLSSVVQDSETLHRLSANKLRTSSKFGPVSIHFIITDWINMYEVALKDATTAIESPFTHARIGMLESAIAALTQHKFAIIYDMPFVQEGIRVLTQYAGWLLPFNVMWNQIQNSSLTPLTRALFIICMIDEYLTETPVHSISELFADTVNLIKDEAFVSIEEAVTNPRTVHESRISSALAYRDPYVFETSPGMLARRLRLDNGIWESNLLSLSTPGIHIEALLHLLNSDPEAETTSGSNVAEHTRGIWEKVQASTSPSMLISTLAESGFTRFSCKLLRRFIAHHTLAGFIHGSVVADEHITDFQQTLGCLALVGGLAYQLVETYAPTTEYVLTYTRTVNETEKRYETLLPALGLPPGGLGQIMRRCFAPRPLIESIQATRVILLNEISHAEARETTYFKQTHNQSSGALLPQAGQSAVREAVLTWFDLRMDSRWGI

SEQ ID NO: 28 - protein, 545 aa, Gallid herpesvirus 2
MSAVTTDEIWPLKVLLDTLRSLSSRTSPTEPWGATATAEARAAIGSFFLASGTMSILQVELTWRDTFSAILEVYKQTRSPEASMLAQNFVGLILWRISVRWDKTSWQENSHRLRRLVAEMTGEEAISWLSRNNLRISAPFGPSVMWPLISEWFAVFEDAANHAFTYTPEHLLSEREFSFNVGDLAASLAHKRFELIYDFPFVQEGIRLVSIASGWIAPFVIMYRCTTNRVFTPLTRILFTIALVDQYFRGLHAPQPFQIKDRFAEDVGALGSKELIPALEANSTKRTSYEVRASAAIAYESPFVHTIQPGMAADKLRNGSDIIMSDTSLTEDSLAIHLSAVLRLISDIGLEEDNGAIDAAKAKLSNSARRAWDAIQYSSSPKQLLEALIERGFVRQVCRAYESALKTYFTRNYGSVDEGDIFDDVQQVVGCVAVIGNVVFGLIESYGPGMTYLSNYMENCVISESDSHFIEALGLERAIISQIIGRCIPPIPHEDYIKAARAVLVAEMDHVASKSEAVGFRQSIRSAKESLMLWFDNRANEIWGI

SEQ ID NO: 29 - protein, 539 aa, Gallid herpesvirus 3
MSETQGEARFPLKTLLDTLRSLSAGTAPLEPWGNATAAEARTAIGSFFQALETMSIQQVESTWRDAFAAVLEVYKQTGSPEAAMLAQNFVGFILWRTSVRWDKMSWKDDSRRLRRLAAEMTGEEAIAWLTRNGLRRSCPFGPSVLWPLISEWLTIFEEIATDAFDYTSEGLLSGRQPAPNALELPASLTQTRFKLIYDFPFVQEGIRLISIAVGWITPFVIMSRCTTNRAFTPLTRILFTLALVDQYFKSPRSPHPSQLKDLFAEDASALGSRELISAVEANNMKRTAYDVRASAAIAYGDPYVYAVQPGMVAEKLRNGPDIILADHALTEDALAIHMSAVVRLITDGDLNDGGGALDAAKAKLSESARRAWGAVQHSSSPRQLLEALIERGFVRQACRVYESALKANLGKTRGTVNELDTFDDVQQVIGNIVFGLMESYGPGMTYLTNYMDNGLPPDADSDFIKVLGLDSAIIAQILGRCIPPNPHEDYVKSARAILAAEMDSAIRQSGAGTANRAIQFAKESLMLWFDSRAEHIWGI

SEQ ID NO: 30 - protein, 544 aa, Meleagrid herpesvirus 1
MSALGKGDNYPLNALLDTLQTLCAENSPTEPWPVTVISEARAAIGTFFLSSTQMSIQQVESTWRDVFSVILEVYQRTKSPEAAMLAQNFTGLILWRVSVRWDKTSWRDESIRLRKLVGEMTGEEPITWLSRNNLRVSASFGPNVMGPLITDWFAEFEDTVTSAVSYTPECLLSERERIPNVWNLTDSLAHKRFELIYDFPFVQEGIRLIARTVGWVVPFVILYRCTTNRAFTPLTRILFTIAFIDQYFRGKGASQHSVLKERFAEDCNALGSEELMSASQANLTKRTSYEVRASAAIAYGDPFIYGIQPGMVAERLRSGEDIIVSSTSLTEDSLAIHISAVLQLISSDGSDHSTSVIDEARTKLSESVRRAWDAIQYSSSPKQLLEALIDNGFVRQSCQAYESALKTYMAKNYRNSVETIFNDLQQVIGCVAVIGNIVFGLIESYGPGMNYLENYVDGSLPPESDSEFIFALGLEHGLISQILGRCIPPDTHDDYVKTTRSVLLAEMDLIARKMDVGGSARALSSARESLLLWFDHRAEVIWGL

SEQ ID NO: 31 - protein, 573 aa, Anatid herpesvirus 1
MDSGDQLSDNEYYDLDEDNTCSDNRSPRPVGRWLLKDMIVALKEIINTQSTPRWTEVEASKVKAIVSTFCLSQEQMTIPQISHSWKEAFDLLLVAFSNTQTPEVAIIIENFTGLVIWRLVVSWDRNTVKADVTKLMALVRDLTSEHVTQSLTRQNLRLSTSYGVSAMRGILLSWLTTFEAAVTTVLATTPDVLLDSERLGFRKDRVPFTSRYIRIIYDFPFVQEGLRFLHRNANWMIPFKIMTRCASDTIYSPLVRTIYTISLVDQYFWGAGRSRPKRLVDQFVKDTDLLGDAELMSPGEANSTKRTSWEVRLSAALAYQDPFVREVQPGMASVRVRTSPDMVLRGGPVFGPALCIHSAAVLNVISGSKQDEFDLGRLNQAAKTTITEAARAAWDTIQHSNTPQQVIDALISTGFVAQNCRNYEVALTSMYSRATTDNGYALNDTQQVIGCVSMVGNVVFGLIDSYGRDADYIDAYAEAMSSLESDSGDFLSAIGLPKGGIEQTIRHCMAPRPITDYIRAARQALVQEIETASSIYKGRLSSRLQTHHTSTHNSVRGSLLLWFDFRAKQIWGI

SEQ ID NO: 32 - protein, 636 aa, Macacine herpesvirus 1
MVSPTPTPPPKEGRAATPPKEGRAATPPRDDRAPPVPKDNTAATPSDNARTTPSTKEDGAAAPPPAAPPGDGRAPSPSGNSRPGHPTDGPLQSLLGALASLAAAGPASPAETPRDADEDSVLLAAKLRAAIAAFLLSTAPIRVVDARTHWRPLLERLCDLHGAHGLPETALLAENLPGLLAHRLAVALPDDPERAFEAMDDLKAGVLATTSPEATRLLEAAGLRTAAALGPARTRQCVTEWTDRWRSVSESCLRLDPRAASGAPADASPPVSPIPLGQPGAGLTTPAYSTIFPAPFVQEGLRFLARASNWATLFSTHLQRVDDATLTPLTRALFTLALVDEYLTTRDRGIVAPPRLLEQFEHTVREIDPAIMIPPIEANKMVRTREEVRVSAALNHLTPRSARAPPGTLMTRVRTDAAVFDPEEPLLSSSALAIFQPAVAALLGSGEPPSAGAQRRLLALLHQTWALIQNTGSPSVVINALIDAGFTPLHCSHYLSALEGFLATGGASRGLAGPGLSEIQQLFGCIALTGANVFALAREYGYHSGYVRAFRRIQDACEKAHARLCEAAGLTGGVLSQTLARVMGPVTPTEHLASLRRALVGEFESAERRFGAGRASPLRETVLIWVDVYGQTEWDI

SEQ ID NO: 33 - protein, 655 aa, Papiine herpesvirus 2
MVSPTPTPPTEENRSRPAPPPKEARGSAATSPKETRSRTTPPPKEARGSAATSPENVRTAPAPGDTRAAAPPTPEETRAPPPPATPPEDVRAATPSGDARLGPPPDGPLQSLLGALTSLATARPAPPTEASGEAGEDAVLLAARLRAAIAAFLLSGAPIRVADARTHWRPLLERLCALHGAHGLPETALLAENLPGLLAHRLAVALPDAPDRAFEAMDHLRAAVLDAASPEATRLLEAAGLRTAAALGPARTRQCVAEWTDRWRSVTESCLRLDPRASSAAPGGADPPVSPVPLGQPSAGLATPAYSPIFPAPFVQEGLRFLARASNWATLFSTHLQSVDDATLTPLTRALFTLSLVDEYLTTRDRGIVAPPRLLEQFERTVREIDPAIMIPPIEANKMVRSREEVRVSAALNHLTPRSARAPPGTLMSRVRTDAAVFDPEEPFLSASALAIFQPAVAALLGSGEPPSAGAQRRLLALLHQTWALIQNTGSPSVVINALIDAGFTPLHCSHYLSALEGFLAAGGAARGLAGPPALSEVQQLFGCVALTGANVFALAREYGYHSGYVRAFRRVQDACEQAHARLCEAAGLAGGVLSQTLARVMGPVTPTEHLASLRRALVGEFESAERRFGAGRPSPLRETVLIWIDVYGQTEWDI

SEQ ID NO: 34 - protein, 570 aa, Human herpesvirus 2
MSDSALQVPAPAGMTPPSAPPPNGPLQVLLGSLTNLRRPPSPSSEPAGSADEPAFLSAAKLHAATAAFLLSGAAVGPAEARACWHPLLEQLCALHRAHGLPETALLAENLPGLLVHRMAVALPETPEAAFREMDVIKDTVLAITGSDTTHALEAAGLRTTAALGPVRVRQCAVEWIDRWRTVTQSCLAMNPRTSLEALGEMSLKMSPVPLGQPGANLTTPAYSLLFPSPIVQEGLRFLALVSNWVTLFSAHLQRIDDAALTPLTRALFTLALVDDYLTTPDRGAVVPPPLLAQFQHTVREIDPAIMIPPLEATKMVRSREEVRVSTALSRVSPRSACAPPGTLMARVRTDAAVFDPDVPFLSASALAIFRPAVTGLLQLGEPPSAGAQQRLLALLQQTWALVQNSNSPSVVINTLTDAGFTPAHCTQYISALEGFLVAGVPARTPPGHGLSEIQQLFGCIALAGANVFGLAREYGHYAGYVKTFRRIQGASEHTHGRLCEAVGLSGGVLSQTLARIMGPAVPTEHLASLRRTLVGEFETAERRFSAGQPSLLRETALIWLDVYGQTHWDL

SEQ ID NO: 35 - protein, 570 aa, Human herpesvirus 1
MADRGLPSEAPVVTTSPAGPPSDGPMQRLLASLAGLRQPPTPTAETANGADDPAFLATAKLRAAMAAFLLSGTAIAPADARDCWRPLLEHLCALHRAHGLPETALLAENLPGLLVHRLVVALPEAPDQAFREMEVIKDTILAVTGSDTSHALDSAGLRTAAALGPVRVRQCAVEWIDRWQTVTKSCLAMSPRTSIEALGETSLKMAPVPLGQPSANLTTPAYSLLFPAPFVQEGLRFLALVSNRVTLFSAHLQRIDDATLTPLTRALFTLALVDEYLTTPERGAVVPPPLLAQFQHTVREIDPAIMIPPLEANKMVRSREEVRVSTALSRVSPRSACAPPGTLMARVRTDVAVFDPDVPFLSSSALAVFQPAVSSLLQLGEQPSAGAQQRLLALLQQTWTLIQNTNSPSVVINTLIDAGFTPSHCTHYLSALEGFLAAGVPARTPTGHGLGEVQQLFGCIALAGSNVFGLAREYGYYANYVKTFRRVQGASEHTHGRLCEAVGLSGGVLSQTLARIMGPAVPTEHLASLRRALVGEFETAERRFSSGQPSLLRETALIWIDVYGQTHWDI

SEQ ID NO: 36 - protein, 612 aa, Saimiriine herpesvirus 1
MTQATRTRVPVEWHELIAAAENDLREHAPAPSHVGSIWNLVDTLEPLATQLREMSRAATAAAPPRLSPGAAGRKLVGHGSAYPPEQTFLLVARLRAAFASFLLAPTAAAPEHVRSGWPRLISLLCELHRGLSLTETALLLENLPGLAVHHIDVAVPRDRAGACRDMSAVIACVRKMAGPETVDALEELGLRTSSPLGPISTQRNVLDWVQRWLAVTKSMHEADPRESADFSSAPPLKNLATLPLGQPGAGLAAPKYHLIFGAPFVQRGLRHLAEVGNRVCVVGAYLRRADDAALTPLARALFTLALVDEHVPSGGGVPSLLVQRFRRDVALVDPTIMIPPLEANPMPRTRGEVRISSALSTRTPGVTCAPPGTLITRVRTDSDVFGTHPEHVSASALAVFQPAVSSLLQAGETEATPEVRQRMLGLLHETWARLQNTTSADVALATLVDAGFTPANCAAYLSALEGFLASGHLVASADSGEKDARGLDGRELGEIQQLFGCISILGRGIFQLAREYGPHAEYVKTFKRIQAACEQRHAQLSHAAGLSQGVLGQALARIMSPTTPTEHLAALRRALVDEFEVAERRFNEGHPSLLREPVMAWVDIYGQTAWDV